European Patent Application EP 4 310 099 A1, published January 24, 2024. Title: Pharmaceutical composition for improving acute lung injury and acute exacerbation of pulmonary fibrosis. Applicant: MIE UNIVERSITY The Board of Trustees of The University Of Illinois. The sequence listing filed with the application follows.

SEQUENCE LISTING (97 sequences)

SEQ ID NO: 1 - protein, 19 aa, Staphylococcus nepalensis
IVMPESSGNPNAVNPAGYR

SEQ ID NO: 2 - DNA, 21 bp, Artificial Sequence
  Primer
tacgaagaactacggctggac

SEQ ID NO: 3 - DNA, 22 bp, Artificial Sequence
  Primer
ggtgtgatcgtctaatgggtca

SEQ ID NO: 4 - DNA, 22 bp, Artificial Sequence
  Primer
gttcagtggttcttactccagc

SEQ ID NO: 5 - DNA, 22 bp, Artificial Sequence
  Primer
actgtaggggttagtcctcgat

SEQ ID NO: 6 - DNA, 23 bp, Artificial Sequence
  Primer
tttccgtggctcttattcaaact

SEQ ID NO: 7 - DNA, 23 bp, Artificial Sequence
  Primer
gcacagtggtaggaacttctcat

SEQ ID NO: 8 - DNA, 23 bp, Mus musculus
tatcagacaccatatacccgagg

SEQ ID NO: 9 - DNA, 21 bp, Artificial Sequence
  Primer
tggggttaggtgagcatagtc

SEQ ID NO: 10 - DNA, 21 bp, Artificial Sequence
  Primer
aggaccaccgcatctctacat

SEQ ID NO: 11 - DNA, 21 bp, Artificial Sequence
  Primer
aagtctggctcgttctcagtg

SEQ ID NO: 12 - DNA, 21 bp, Artificial Sequence
  Primer
tgcacagtttccttgtacgga

SEQ ID NO: 13 - DNA, 22 bp, Artificial Sequence
  Primer
gagcttgggtctcctgatagaa

SEQ ID NO: 14 - DNA, 20 bp, Artificial Sequence
  Primer
gctctgaggagttgcgtctg

SEQ ID NO: 15 - DNA, 22 bp, Mus musculus
cacactgtggacaaagtctctt

SEQ ID NO: 16 - DNA, 21 bp, Artificial Sequence
  Primer
gcgctcagaaagacactacag

SEQ ID NO: 17 - DNA, 20 bp, Artificial Sequence
  Primer
cctcttgcagacgccttagc

SEQ ID NO: 18 - DNA, 21 bp, Artificial Sequence
  Primer
ggagcgagatccctccaaaat

SEQ ID NO: 19 - DNA, 23 bp, Artificial Sequence
  Primer
ggctgttgtcatacttctcatgg

SEQ ID NO: 20 - DNA, 20 bp, Artificial Sequence
  Primer
gccttctttgagttcggtgg

SEQ ID NO: 21 - DNA, 19 bp, Mus musculus
atctcccggttgacgctct

SEQ ID NO: 22 - DNA, 21 bp, Mus musculus
cccgagaggtctttttccgag

SEQ ID NO: 23 - DNA, 21 bp, Artificial Sequence
  Primer
ccagcccatgatggttctgat

SEQ ID NO: 24 - DNA, 22 bp, Artificial Sequence
  Primer
gactgaatcggagatggagacc

SEQ ID NO: 25 - DNA, 20 bp, Artificial Sequence
  Primer
gcagttcaaactcgtcgcct

SEQ ID NO: 26 - DNA, 21 bp, Artificial Sequence
  Primer
gtcaccatacatggaatggca

SEQ ID NO: 27 - DNA, 20 bp, Artificial Sequence
  Primer
ctgatccaaccgtgtgcaaa

SEQ ID NO: 28 - DNA, 20 bp, Artificial Sequence
  Primer
caatgaccccgcacgatttc

SEQ ID NO: 29 - DNA, 19 bp, Artificial Sequence
  Primer
catggagggcggattggaa

SEQ ID NO: 30 - DNA, 22 bp, Artificial Sequence
  Primer
acactaagggccgaagataacg

SEQ ID NO: 31 - DNA, 22 bp, Artificial Sequence
  Primer
acagcatctccaatatggctga

SEQ ID NO: 32 - DNA, 21 bp, Artificial Sequence
  Primer
agaagaagtggtgcttcggaa

SEQ ID NO: 33 - DNA, 21 bp, Artificial Sequence
  Primer
agtttgcgtggcctgtactaa

SEQ ID NO: 34 - DNA, 22 bp, Artificial Sequence
  Primer
catggaagcgaatcaatggact

SEQ ID NO: 35 - DNA, 21 bp, Artificial Sequence
  Primer
ctgtaccagaccgagatgtca

SEQ ID NO: 36 - protein, 121 aa, Mus musculus
EVQVLESGGGLVQPGNSLKLSCATSGFTFSTAWMYWYRQFPEKRLEWVARIKAKSNSYATDYTESVKGRFTISRDDSKGSIYLRMNNLKEEDTAIYYCASTDAFYFSHSYWGQGVLVTVSS

SEQ ID NO: 37 - protein, 8 aa, Mus musculus
GFTFSTAW

SEQ ID NO: 38 - protein, 10 aa, Mus musculus
IKAKSNSYAT

SEQ ID NO: 39 - protein, 12 aa, Mus musculus
ASTDAFYFSHSY

SEQ ID NO: 40 - protein, 113 aa, Mus musculus
DIVMTQTPSSQAVSAGEKVTMRCRSSQSLLYSENKKNYLAWYQQKPGRSPKLLIYWASTGESGVPDRFIGSGSGTDFTLTISSVQAEDLAVYYCQQYYNFPLTFGSGTKLEIK

SEQ ID NO: 41 - protein, 12 aa, Mus musculus
QSLLYSENKKNY

SEQ ID NO: 42 - protein, 4 aa, Mus musculus
WAST

SEQ ID NO: 43 - protein, 9 aa, Mus musculus
QQYYNFPLT

SEQ ID NO: 44 - protein, 113 aa, Mus musculus
DIVMTQSPSSQAVSAGEKVTMSCKSSQNLLYSEDKKNYLAWYQQKPGQSPKLLIYWASTRESGVPDRFIGSGSGTDFTLTVTSVQAEDLAVYYCQQYYNFPRTFGGGTKLELK

SEQ ID NO: 45 - protein, 12 aa, Mus musculus
QNLLYSEDKKNY

SEQ ID NO: 46 - protein, 3 aa, Mus musculus
WAS

SEQ ID NO: 47 - protein, 9 aa, Mus musculus
QQYYNFPRT

SEQ ID NO: 48 - protein, 118 aa, Mus musculus
EVKLVESGGGLVQPGNSLTLSCVASGFTFTNYGMHWIRQAPKKGLEWIAMIYYDSSKMSYADTVKGRFTISRDNSKNTLYLEMNSLRSEDTAMYYCAAEGFGTPFPYWGQGTLVTVSS

SEQ ID NO: 49 - protein, 8 aa, Mus musculus
IYYDSSKM

SEQ ID NO: 50 - protein, 11 aa, Mus musculus
AAEGFGTPFPY

SEQ ID NO: 51 - protein, 227 aa, Mus musculus
MESQTQVLMSLLLWVSGSCGDIVMTQTPSSRAVSAGEKVTMSCKSSQSLLYSENEKNYLAWYQQRPGQSPKLLIYWASTRESGVPDRFIGTGSGTDFTLTISSVQAEDLAVYYCQQYYHFPRTFGGGTRLELKRADAAPTVSIFPPSMEQLTSGGATVVCFVNNFYPRDISVKWKIDGSEQRDGVLDSVTDQDSKDSTYSMSSTLSLTKVEYERHNLYTCEVVHKTS

SEQ ID NO: 52 - protein, 12 aa, Mus musculus
QSLLYSENEKNY

SEQ ID NO: 53 - protein, 3 aa, Mus musculus
WAS

SEQ ID NO: 54 - protein, 9 aa, Mus musculus
QQYYHFPRT

SEQ ID NO: 55 - protein, 19 aa, Artificial Sequence
  Primer
IVMPESSGNPNAVSPAGYR

SEQ ID NO: 56 - protein, 19 aa, Artificial Sequence
  Primer
IVMPESSGNPNAVNAAGYR

SEQ ID NO: 57 - protein, 19 aa, Artificial Sequence
  Primer
IVMPESSGNPNAVNPNGYR

SEQ ID NO: 58 - protein, 19 aa, Staphylococcus
IVMPESGGNPNAVNPAGYR

SEQ ID NO: 59 - protein, 19 aa, Staphylococcus
IIMPESGGNPNIVNPYGYS

SEQ ID NO: 60 - protein, 19 aa, Staphylococcus
IVMPESGGNPNAVNPYGYR

SEQ ID NO: 61 - protein, 19 aa, Staphylococcus
IVLPESSGNPNAVNPAGYR

SEQ ID NO: 62 - protein, 19 aa, Staphylococcus
IVLPESSGNPNAVNELGYR

SEQ ID NO: 63 - protein, 19 aa, Staphylococcus
IVMPESGGNPNAVNELGYR

SEQ ID NO: 64 - protein, 19 aa, Staphylococcus
IVMPESSGNPNAVNELGYR

SEQ ID NO: 65 - protein, 19 aa, Staphylococcus
IVMPESSGNPDAVNELGYR

SEQ ID NO: 66 - protein, 19 aa, Staphylococcus
IAQRESGGDLKAVNPSSGA

SEQ ID NO: 67 - protein, 19 aa, Staphylococcus
IAERESGGDLKAVNPSSGA

SEQ ID NO: 68 - protein, 7 aa, Artificial Sequence
  Artificial
PESSGNP

SEQ ID NO: 69 - protein, 5 aa, Artificial Sequence
  Artificial
NPAGY

SEQ ID NO: 70 - protein, 8 aa, Mus musculus
GFTFTNYG

SEQ ID NO: 71 - protein, 118 aa, Mus musculus
EVKLVESGGGLVQPGNSLTLSCGASGFTFTNYGMHWIRQAPKKGLEWIGMIYYDSSKMSYADTVKGRFTISRDNSKNILYLEMNSLRSEDTAMYYCAAEGFGTPFPYWGQGTLVTVSS

SEQ ID NO: 72 - protein, 5 aa, Mus musculus
NYGMH

SEQ ID NO: 73 - protein, 17 aa, Mus musculus
MIYYDSSKMSYADTVKG

SEQ ID NO: 74 - protein, 9 aa, Mus musculus
EGFGTPFPY

SEQ ID NO: 75 - protein, 113 aa, Mus musculus
DIVMTQTPSSQAVSAGEKVTMSCKSSQSLLYREDTKNYLAWYQQRPGQSPKLLIYWASTRESGVPDRFIGSGSGTDFTLTISSVQAEDLAVYYCQQYYHFPRTFGGGTRLELK

SEQ ID NO: 76 - protein, 17 aa, Mus musculus
KSSQSLLYREDTKNYLA

SEQ ID NO: 77 - protein, 7 aa, Mus musculus
WASTRES

SEQ ID NO: 78 - protein, 9 aa, Mus musculus
QQYYHFPRT

SEQ ID NO: 79 - protein, 226 aa, Mus musculus
MELCMMWIFLVAFLKGVQCEVQVLESGGGLVQPGNSLKLSCATSGFTFSTAWMYWYRQFPEKRLEWVARIKAKSNSYATDYTESVKGRFTISRDDSKGSIYLRMNNLKEEDTAIYYCASTDAFYFSHSYWGQGVLVTVSSAETTAPSVYPLAPGTALKSNSMVTLGCLVKGYFPEPVTVTWNSGALSSGVHTFPAVLQSGLYTLTSSVTVPSSTWSSQAVTCNVAH

SEQ ID NO: 80 - protein, 19 aa, Artificial Sequence
  Artificial
MELCMMWIFLVAFLKGVQC

SEQ ID NO: 81 - protein, 86 aa, Artificial Sequence
  Artificial
AETTAPSVYPLAPGTALKSNSMVTLGCLVKGYFPEPVTVTWNSGALSSGVHTFPAVLQSGLYTLTSSVTVPSSTWSSQAVTCNVAH

SEQ ID NO: 82 - protein, 227 aa, Mus musculus
MESQTQVLMSLLLWVSGTCGDIVMTQTPSSQAVSAGEKVTMRCRSSQSLLYSENKKNYLAWYQQKPGRSPKLLIYWASTGESGVPDRFIGSGSGTDFTLTISSVQAEDLAVYYCQQYYNFPLTFGSGTKLEIKRADAAPTVSIFPPSMEQLTSGGATVVCFVNNFYPRDISVKWKIDGSEQRDGVLDSVTDQDSKDSTYSMSSTLSLTKVEYERHNLYTCEVVHKTS

SEQ ID NO: 83 - protein, 20 aa, Artificial Sequence
  Artificial
MESQTQVLMSLLLWVSGTCG

SEQ ID NO: 84 - protein, 94 aa, Artificial Sequence
  Artificial
RADAAPTVSIFPPSMEQLTSGGATVVCFVNNFYPRDISVKWKIDGSEQRDGVLDSVTDQDSKDSTYSMSSTLSLTKVEYERHNLYTCEVVHKTS

SEQ ID NO: 85 - protein, 227 aa, Mus musculus
MESQTQVLMSLLLWVSGTCGDIVMTQSPSSQAVSAGEKVTMSCKSSQNLLYSEDKKNYLAWYQQKPGQSPKLLIYWASTRESGVPDRFIGSGSGTDFTLTVTSVQAEDLAVYYCQQYYNFPRTFGGGTKLELKRADAAPTVSIFPPSMEQLTSGGATVVCFVNNFYPRDISVKWKIDGSEQRDGVLDSVTDQDSKDSTYSMSSTLSLTKVEYERHNLYTCEVVHKTS

SEQ ID NO: 86 - protein, 20 aa, Artificial Sequence
  Artificial
MESQTQVLMSLLLWVSGTCG

SEQ ID NO: 87 - protein, 94 aa, Artificial Sequence; identical to SEQ ID NO: 84
  Artificial

SEQ ID NO: 88 - protein, 221 aa, Mus musculus
MDFRLNLVFLVFILKGVWCEVKLVESGGGLVQPGNSLTLSCVASGFTFTNYGMHWIRQAPKKGLEWIAMIYYDSSKMSYADTVKGRFTISRDNSKNTLYLEMNSLRSEDTAMYYCAAEGFGTPFPYWGQGTLVTVSSAQTTAPSVYPLAPGCGDTTSSTVTLGCLVKGYFPEPVTVTWNSGALSSDVHTFPAVLQSGLYTLTSSVTSSTWPSQTVTCNVAH

SEQ ID NO: 89 - protein, 19 aa, Artificial Sequence
  Artificial
MDFRLNLVFLVFILKGVWC

SEQ ID NO: 90 - protein, 84 aa, Artificial Sequence
  Artificial
AQTTAPSVYPLAPGCGDTTSSTVTLGCLVKGYFPEPVTVTWNSGALSSDVHTFPAVLQSGLYTLTSSVTSSTWPSQTVTCNVAH

SEQ ID NO: 91 - protein, 227 aa, Mus musculus; identical to SEQ ID NO: 51

SEQ ID NO: 92 - protein, 20 aa, Artificial Sequence
  Artificial
MESQTQVLMSLLLWVSGSCG

SEQ ID NO: 93 - protein, 94 aa, Artificial Sequence; identical to SEQ ID NO: 84
  Artificial

SEQ ID NO: 94 - protein, 137 aa, Mus musculus
MDFRLNLVFLVFILKGVWCEVKLVESGGGLVQPGNSLTLSCGASGFTFTNYGMHWIRQAPKKGLEWIGMIYYDSSKMSYADTVKGRFTISRDNSKNILYLEMNSLRSEDTAMYYCAAEGFGTPFPYWGQGTLVTVSS

SEQ ID NO: 95 - protein, 18 aa, Artificial Sequence
  Artificial
MDFRLNLVFLVFILKGVW

SEQ ID NO: 96 - protein, 133 aa, Mus musculus
MESQTQVLMSLLLWVSGTYGDIVMTQTPSSQAVSAGEKVTMSCKSSQSLLYREDTKNYLAWYQQRPGQSPKLLIYWASTRESGVPDRFIGSGSGTDFTLTISSVQAEDLAVYYCQQYYHFPRTFGGGTRLELK

SEQ ID NO: 97 - protein, 20 aa, Artificial Sequence
  Artificial
MESQTQVLMSLLLWVSGTYG